European Patent Application EP 4 653 051 A2, published November 26, 2025. Title: HUMAN ANTIBODIES TO EBOLA VIRUS GLYCOPROTEIN. Applicant: Regeneron Pharmaceuticals, Inc. Application EP. The sequence listing filed with the application follows.

SEQUENCE LISTING (318 sequences)

SEQ ID NO: 1 - DNA, 342 bp, synthetic construct
  misc_feature 1..342: note = synthetic
  source 1..342: mol_type = other DNA
cagctgcagctgcaggagtcgggcccaggactggtgaagccttcggagaccctgtccctcacctgcactgtctctggtggctccatcagcagtagtagttactactggggctggatccgccagcccccagggaaggggctggagtggattgggagtatctattatgatggggacacctactacaacccgtccctcaagagtcgagtcaccatatccgtagacacgtccaagaaccagttctccctgaggctgagctctgtgaccgccgcagacacggcagtgtattactgtgcgagacagtttgactactggggccagggaaccctggtcaccgtctcctca

SEQ ID NO: 2 - protein, 114 aa, synthetic construct
  REGION 1..114: note = synthetic
QLQLQESGPGLVKPSETLSLTCTVSGGSISSSSYYWGWIRQPPGKGLEWIGSIYYDGDTYYNPSLKSRVTISVDTSKNQFSLRLSSVTAADTAVYYCARQFDYWGQGTLVTVSS

SEQ ID NO: 3 - DNA, 30 bp, synthetic construct
  misc_feature 1..30: note = synthetic
  source 1..30: mol_type = other DNA
ggtggctccatcagcagtagtagttactac

SEQ ID NO: 4 - protein, 10 aa, synthetic construct
  REGION 1..10: note = synthetic
GGSISSSSYY

SEQ ID NO: 5 - DNA, 21 bp, synthetic construct
  misc_feature 1..21: note = synthetic
  source 1..21: mol_type = other DNA
atctattatgatggggacacc

SEQ ID NO: 6 - protein, 7 aa, synthetic construct
  REGION 1..7: note = synthetic
IYYDGDT

SEQ ID NO: 7 - DNA, 18 bp, synthetic construct
  misc_feature 1..18: note = synthetic
  source 1..18: mol_type = other DNA
gcgagacagtttgactac

SEQ ID NO: 8 - protein, 6 aa, synthetic construct
  REGION 1..6: note = synthetic
ARQFDY

SEQ ID NO: 9 - DNA, 321 bp, synthetic construct
  misc_feature 1..321: note = synthetic
  source 1..321: mol_type = other DNA
gaaatagtgatgacgcagtctccagccaccctgtctgtgtctccaggggaaagagccaccctctcctgcagggccagtcagagtgttagtagcaacttagcctggtaccagcagaaacctggccaggctcccaggctcctcatctatggtgcatccaccagggccactggtatcccagccaggttcagtggcagtgggtctgggacagagttcactctcaccatcagcagcctgcagtctgaagattttgcagtttattactgtcagcagtataaaaactggccgatcaccttcggccaagggacacgactggagattaaa

SEQ ID NO: 10 - protein, 107 aa, synthetic construct
  REGION 1..107: note = synthetic
EIVMTQSPATLSVSPGERATLSCRASQSVSSNLAWYQQKPGQAPRLLIYGASTRATGIPARFSGSGSGTEFTLTISSLQSEDFAVYYCQQYKNWPITFGQGTRLEIK

SEQ ID NO: 11 - DNA, 18 bp, synthetic construct
  misc_feature 1..18: note = synthetic
  source 1..18: mol_type = other DNA
cagagtgttagtagcaac

SEQ ID NO: 12 - protein, 6 aa, synthetic construct
  REGION 1..6: note = synthetic
QSVSSN

SEQ ID NO: 13-14 - skipped (2 entries)

SEQ ID NO: 15 - DNA, 27 bp, synthetic construct
  misc_feature 1..27: note = synthetic
  source 1..27: mol_type = other DNA
cagcagtataaaaactggccgatcacc

SEQ ID NO: 16 - protein, 9 aa, synthetic construct
  REGION 1..9: note = synthetic
QQYKNWPIT

SEQ ID NO: 17 - DNA, 354 bp, synthetic construct
  misc_feature 1..354: note = synthetic
  source 1..354: mol_type = other DNA
gaggtgcagctggtggagtctgggggaggcttggtacagcctggggggtccctgagactctcctgtgcagcctctggattcaccttcagtagctacgacatgcactgggtccgccaagctacaggaaaaggtctggagtgggtctcagctattggtactgctggtgacacatactatccaggctccgtgaagggccgattcaccatctccagagaaaatgccaaaaactccttgtatcttcaaatgaacagcctgagagccggggacacggctgtgtattactgtgcaagaacatggttcggggagctttactttgactactggggccagggaaccctggtcaccgtctcctca

SEQ ID NO: 18 - protein, 118 aa, synthetic construct
  REGION 1..118: note = synthetic
EVQLVESGGGLVQPGGSLRLSCAASGFTFSSYDMHWVRQATGKGLEWVSAIGTAGDTYYPGSVKGRFTISRENAKNSLYLQMNSLRAGDTAVYYCARTWFGELYFDYWGQGTLVTVSS

SEQ ID NO: 19 - DNA, 24 bp, synthetic construct
  misc_feature 1..24: note = synthetic
  source 1..24: mol_type = other DNA
ggattcaccttcagtagctacgac

SEQ ID NO: 20 - protein, 8 aa, synthetic construct
  REGION 1..8: note = synthetic
GFTFSSYD

SEQ ID NO: 21 - DNA, 21 bp, synthetic construct
  misc_feature 1..21: note = synthetic
  source 1..21: mol_type = other DNA
attggtactgctggtgacaca

SEQ ID NO: 22 - protein, 7 aa, synthetic construct
  REGION 1..7: note = synthetic
IGTAGDT

SEQ ID NO: 23 - DNA, 36 bp, synthetic construct
  misc_feature 1..36: note = synthetic
  source 1..36: mol_type = other DNA
gcaagaacatggttcggggagctttactttgactac

SEQ ID NO: 24 - protein, 12 aa, synthetic construct
  REGION 1..12: note = synthetic
ARTWFGELYFDY

SEQ ID NO: 25 - DNA, 339 bp, synthetic construct
  misc_feature 1..339: note = synthetic
  source 1..339: mol_type = other DNA
gacatcgtgatgacccagtctccagactccctggctgtgtctctgggcgagagggccaccatcaactgcaagtccagccagagtgttttatacagctccaacaataagaactacttagcttggtaccagcagaaaccaggacagcctcctaagctgctcatttactgggcatctacccgggaatccggggtccctgaccgattcagtggcagcgggtctgggacagaattcactctcaccatcaccagcctgcaggctgaagatgtggcagtttattactgtcagcaatattatagtagtccgctcactttcggcggagggaccaaggtggagatcaaa

SEQ ID NO: 26 - protein, 113 aa, synthetic construct
  REGION 1..113: note = synthetic
DIVMTQSPDSLAVSLGERATINCKSSQSVLYSSNNKNYLAWYQQKPGQPPKLLIYWASTRESGVPDRFSGSGSGTEFTLTITSLQAEDVAVYYCQQYYSSPLTFGGGTKVEIK

SEQ ID NO: 27 - DNA, 36 bp, synthetic construct
  misc_feature 1..36: note = synthetic
  source 1..36: mol_type = other DNA
cagagtgttttatacagctccaacaataagaactac

SEQ ID NO: 28 - protein, 12 aa, synthetic construct
  REGION 1..12: note = synthetic
QSVLYSSNNKNY

SEQ ID NO: 29-30 - skipped (2 entries)

SEQ ID NO: 31 - DNA, 27 bp, synthetic construct
  misc_feature 1..27: note = synthetic
  source 1..27: mol_type = other DNA
cagcaatattatagtagtccgctcact

SEQ ID NO: 32 - protein, 9 aa, synthetic construct
  REGION 1..9: note = synthetic
QQYYSSPLT

SEQ ID NO: 33 - DNA, 375 bp, synthetic construct
  misc_feature 1..375: note = synthetic
  source 1..375: mol_type = other DNA
gaggtgcagctggtggagtctgggggaggcttggtacagcctggggggtccctgagactctcctgtgcagcctctggattcacctttagcagctatgccatgacctgggtccgccaggctccagggaagggcctggagtgggtctcaagtattagtggtagtggtactagcacatactacgcagactccgtgaagggccggttcaccatctccagagacaattccaagaacacactgtatctgcaaatgaacagcctgcgagccgaggacacggccctatattactgttcgagagatatatatacctggaacttcctctcactaattggcggtatggacgtctggggccaagggaccacggtcaccgtctcctca

SEQ ID NO: 34 - protein, 125 aa, synthetic construct
  REGION 1..125: note = synthetic
EVQLVESGGGLVQPGGSLRLSCAASGFTFSSYAMTWVRQAPGKGLEWVSSISGSGTSTYYADSVKGRFTISRDNSKNTLYLQMNSLRAEDTALYYCSRDIYTWNFLSLIGGMDVWGQGTTVTVSS

SEQ ID NO: 35 - DNA, 24 bp, synthetic construct
  misc_feature 1..24: note = synthetic
  source 1..24: mol_type = other DNA
ggattcacctttagcagctatgcc

SEQ ID NO: 36 - protein, 8 aa, synthetic construct
  REGION 1..8: note = synthetic
GFTFSSYA

SEQ ID NO: 37 - DNA, 24 bp, synthetic construct
  misc_feature 1..24: note = synthetic
  source 1..24: mol_type = other DNA
attagtggtagtggtactagcaca

SEQ ID NO: 38 - protein, 8 aa, synthetic construct
  REGION 1..8: note = synthetic
ISGSGTST

SEQ ID NO: 39 - DNA, 54 bp, synthetic construct
  misc_feature 1..54: note = synthetic
  source 1..54: mol_type = other DNA
tcgagagatatatatacctggaacttcctctcactaattggcggtatggacgtc

SEQ ID NO: 40 - protein, 18 aa, synthetic construct
  REGION 1..18: note = synthetic
SRDIYTWNFLSLIGGMDV

SEQ ID NO: 41 - DNA, 321 bp, synthetic construct
  misc_feature 1..321: note = synthetic
  source 1..321: mol_type = other DNA
gacatccagatgacccagtctccatcctccctgtctgcatctgtaggagacagagtcaccatcacttgccgggcaagtcagggcattagaattgatttaggctggtatcagcagaaaccagggaaagcccctaaccgcctgatctatgctgcatccagtttgcaaggtggggtcccatcaaggttcagcggcagtggatctgggacagaattcactctcacaatcagcagcctgcagcctgaagattttgcaacttattactgtctacagcaaaatagttacccgtggacgttcggccaagggaccaaggtggaaatcaaa

SEQ ID NO: 42 - protein, 107 aa, synthetic construct
  REGION 1..107: note = synthetic
DIQMTQSPSSLSASVGDRVTITCRASQGIRIDLGWYQQKPGKAPNRLIYAASSLQGGVPSRFSGSGSGTEFTLTISSLQPEDFATYYCLQQNSYPWTFGQGTKVEIK

SEQ ID NO: 43 - DNA, 18 bp, synthetic construct
  misc_feature 1..18: note = synthetic
  source 1..18: mol_type = other DNA
cagggcattagaattgat

SEQ ID NO: 44 - protein, 6 aa, synthetic construct
  REGION 1..6: note = synthetic
QGIRID

SEQ ID NO: 45-46 - skipped (2 entries)

SEQ ID NO: 47 - DNA, 27 bp, synthetic construct
  misc_feature 1..27: note = synthetic
  source 1..27: mol_type = other DNA
ctacagcaaaatagttacccgtggacg

SEQ ID NO: 48 - protein, 9 aa, synthetic construct
  REGION 1..9: note = synthetic
LQQNSYPWT

SEQ ID NO: 49 - DNA, 387 bp, synthetic construct
  misc_feature 1..387: note = synthetic
  source 1..387: mol_type = other DNA
gaggtgcagctggtggagtctgggggaggcttggtacagcctggggggtccctgagactctcctgtgcagcctctggattcacctttagcagctatgccatgaactgggtccgccaggctccagggaaggggctggagtgggtctcagttattagtggtagtggtggttggagaaactacgcagactccgtgaagggccggatcaccatctccagagacaattccaagaacacgctgtatctgcaaatgaacaacctgagagccgaggacacggccgtatattattgtgcgaaagatcggggtgcgacttttggagtggttattttgggacccccctattacggtatggacgtctggggccaagggaccacggtcaccgtctcctca

SEQ ID NO: 50 - protein, 129 aa, synthetic construct
  REGION 1..129: note = synthetic
EVQLVESGGGLVQPGGSLRLSCAASGFTFSSYAMNWVRQAPGKGLEWVSVISGSGGWRNYADSVKGRITISRDNSKNTLYLQMNNLRAEDTAVYYCAKDRGATFGVVILGPPYYGMDVWGQGTTVTVSS

SEQ ID NO: 51 - DNA, 24 bp, synthetic construct
  misc_feature 1..24: note = synthetic
  source 1..24: mol_type = other DNA
ggattcacctttagcagctatgcc

SEQ ID NO: 52 - protein, 8 aa, synthetic construct
  REGION 1..8: note = synthetic
GFTFSSYA

SEQ ID NO: 53 - DNA, 24 bp, synthetic construct
  misc_feature 1..24: note = synthetic
  source 1..24: mol_type = other DNA
attagtggtagtggtggttggaga

SEQ ID NO: 54 - protein, 8 aa, synthetic construct
  REGION 1..8: note = synthetic
ISGSGGWR

SEQ ID NO: 55 - DNA, 66 bp, synthetic construct
  misc_feature 1..66: note = synthetic
  source 1..66: mol_type = other DNA
gcgaaagatcggggtgcgacttttggagtggttattttgggacccccctattacggtatggacgtc

SEQ ID NO: 56 - protein, 22 aa, synthetic construct
  REGION 1..22: note = synthetic
AKDRGATFGVVILGPPYYGMDV

SEQ ID NO: 57 - DNA, 321 bp, synthetic construct
  misc_feature 1..321: note = synthetic
  source 1..321: mol_type = other DNA
gacatccagatgacccagtctccatcctccctgtctgcatctgtaagagacagagtcaccatcacttgccgggcaagtcagagcattagcacttatttaaattggtatcagcagaaaccagggaaagcccctaagctcctgatctatgctgcatccagtttgcaaagtggggtcccatcaaggttcagtggcagtggatctgggacaggtttcactctcaccatcagcagtctgcaacctgaagattttgcaacttactactgtcaacagagttacagtatcccgtacacttttggccaggggaccaagctggagatcaaa

SEQ ID NO: 58 - protein, 107 aa, synthetic construct
  REGION 1..107: note = synthetic
DIQMTQSPSSLSASVRDRVTITCRASQSISTYLNWYQQKPGKAPKLLIYAASSLQSGVPSRFSGSGSGTGFTLTISSLQPEDFATYYCQQSYSIPYTFGQGTKLEIK

SEQ ID NO: 59 - DNA, 18 bp, synthetic construct
  misc_feature 1..18: note = synthetic
  source 1..18: mol_type = other DNA
cagagcattagcacttat

SEQ ID NO: 60 - protein, 6 aa, synthetic construct
  REGION 1..6: note = synthetic
QSISTY

SEQ ID NO: 61-62 - skipped (2 entries)

SEQ ID NO: 63 - DNA, 27 bp, synthetic construct
  misc_feature 1..27: note = synthetic
  source 1..27: mol_type = other DNA
caacagagttacagtatcccgtacact

SEQ ID NO: 64 - protein, 9 aa, synthetic construct
  REGION 1..9: note = synthetic
QQSYSIPYT

SEQ ID NO: 65 - DNA, 354 bp, synthetic construct
  misc_feature 1..354: note = synthetic
  source 1..354: mol_type = other DNA
gaggtgcagctggtggagtctgggggaggcttggtacagcctggggggtccctgagactctcctgtgcagcctctggattcacctctagcagctatgccatgaactgggtccgccaggctccagggaaggggctggagtgggtctcaacaattagtggtatgggtggtagcacatactacgcagactccgtgaagggccggttcaccatctccagagacaattccaagaacacgctgtatctgcaaatgaacagcctgagagccgaggacacggccgtatattactgtgcgaaaaggggatatccccattcttttgatatctggggccaagggacaatggtcaccgtctcttca

SEQ ID NO: 66 - protein, 118 aa, synthetic construct
  REGION 1..118: note = synthetic
EVQLVESGGGLVQPGGSLRLSCAASGFTSSSYAMNWVRQAPGKGLEWVSTISGMGGSTYYADSVKGRFTISRDNSKNTLYLQMNSLRAEDTAVYYCAKRGYPHSFDIWGQGTMVTVSS

SEQ ID NO: 67 - DNA, 24 bp, synthetic construct
  misc_feature 1..24: note = synthetic
  source 1..24: mol_type = other DNA
ggattcacctctagcagctatgcc

SEQ ID NO: 68 - protein, 8 aa, synthetic construct
  REGION 1..8: note = synthetic
GFTSSSYA

SEQ ID NO: 69 - DNA, 24 bp, synthetic construct
  misc_feature 1..24: note = synthetic
  source 1..24: mol_type = other DNA
attagtggtatgggtggtagcaca

SEQ ID NO: 70 - protein, 8 aa, synthetic construct
  REGION 1..8: note = synthetic
ISGMGGST

SEQ ID NO: 71 - DNA, 33 bp, synthetic construct
  misc_feature 1..33: note = synthetic
  source 1..33: mol_type = other DNA
gcgaaaaggggatatccccattcttttgatatc

SEQ ID NO: 72 - protein, 11 aa, synthetic construct
  REGION 1..11: note = synthetic
AKRGYPHSFDI

SEQ ID NO: 73 - DNA, 318 bp, synthetic construct
  misc_feature 1..318: note = synthetic
  source 1..318: mol_type = other DNA
gacatccagatgacccagtctccatcctccctgtctgcatctgtaggagacagagtcaccatcacttgccgggcaagtcagagcattagcagctttttaaattggtatcagcagaaaccagggaaagcccctaaactcctgatctatgctgcatccagtttgcaaagtggggtcccatcaaggttcagtggcagtggatctgggacagatttcactctcaccatcagcagtctgcaacctgaagattttgcaacttactactgtcaacagagttacagtaccctcaccttcggccaagggacacgactggagattaaa

SEQ ID NO: 74 - protein, 106 aa, synthetic construct
  REGION 1..106: note = synthetic
DIQMTQSPSSLSASVGDRVTITCRASQSISSFLNWYQQKPGKAPKLLIYAASSLQSGVPSRFSGSGSGTDFTLTISSLQPEDFATYYCQQSYSTLTFGQGTRLEIK

SEQ ID NO: 75 - DNA, 18 bp, synthetic construct
  misc_feature 1..18: note = synthetic
  source 1..18: mol_type = other DNA
cagagcattagcagcttt

SEQ ID NO: 76 - protein, 6 aa, synthetic construct
  REGION 1..6: note = synthetic
QSISSF

SEQ ID NO: 77-78 - skipped (2 entries)

SEQ ID NO: 79 - DNA, 24 bp, synthetic construct
  misc_feature 1..24: note = synthetic
  source 1..24: mol_type = other DNA
caacagagttacagtaccctcacc

SEQ ID NO: 80 - protein, 8 aa, synthetic construct
  REGION 1..8: note = synthetic
QQSYSTLT

SEQ ID NO: 81 - DNA, 354 bp, synthetic construct
  misc_feature 1..354: note = synthetic
  source 1..354: mol_type = other DNA
gaggtgcagctggtggagtctgggggaggcttggtacagcctggggggtccctgagactctcctgtgcagcctctgaattcacctttagcagctatgccatgagctgggtccgccaggctccagggaaggggctggagtgggtctcagctattagtggtagtagtggtagcacatactacgcagactccgtgaagggccggttcaccatctccagagacaattccaaaaagacgctgtatctacaaatgaacagcctgagagtcgaggacacggccgtatattactgtgcgaaaggggggtacccccattcttttgatatctggggccatgggacaatggtcaccgtctcttca

SEQ ID NO: 82 - protein, 118 aa, synthetic construct
  REGION 1..118: note = synthetic
EVQLVESGGGLVQPGGSLRLSCAASEFTFSSYAMSWVRQAPGKGLEWVSAISGSSGSTYYADSVKGRFTISRDNSKKTLYLQMNSLRVEDTAVYYCAKGGYPHSFDIWGHGTMVTVSS

SEQ ID NO: 83 - DNA, 24 bp, synthetic construct
  misc_feature 1..24: note = synthetic
  source 1..24: mol_type = other DNA
gaattcacctttagcagctatgcc

SEQ ID NO: 84 - protein, 8 aa, synthetic construct
  REGION 1..8: note = synthetic
EFTFSSYA

SEQ ID NO: 85 - DNA, 24 bp, synthetic construct
  misc_feature 1..24: note = synthetic
  source 1..24: mol_type = other DNA
attagtggtagtagtggtagcaca

SEQ ID NO: 86 - protein, 8 aa, synthetic construct
  REGION 1..8: note = synthetic
ISGSSGST

SEQ ID NO: 87 - DNA, 33 bp, synthetic construct
  misc_feature 1..33: note = synthetic
  source 1..33: mol_type = other DNA
gcgaaaggggggtacccccattcttttgatatc

SEQ ID NO: 88 - protein, 11 aa, synthetic construct
  REGION 1..11: note = synthetic
AKGGYPHSFDI

SEQ ID NO: 89 - DNA, 318 bp, synthetic construct
  misc_feature 1..318: note = synthetic
  source 1..318: mol_type = other DNA
gacatccagatgacccagtctccatcctccctgtctgcatctgtaggagacagagtcaccatcacttgccgggcaagtcagagcattagcagctttttaaattggtatcagcagaaaccagggaaagcccctaaactcctgatctatgctgcatccagtttgcaaagtggggtcccatcaaggttcagtggcagtggatctgggacagatttcactctcaccatcagcagtctgcaacctgaagattttgcaacttactactgtcaacagagttacagttccatcaccttcggccaagggacacgactggagattaaa

SEQ ID NO: 90 - protein, 106 aa, synthetic construct
  REGION 1..106: note = synthetic
DIQMTQSPSSLSASVGDRVTITCRASQSISSFLNWYQQKPGKAPKLLIYAASSLQSGVPSRFSGSGSGTDFTLTISSLQPEDFATYYCQQSYSSITFGQGTRLEIK

SEQ ID NO: 91 - DNA, 18 bp, synthetic construct
  misc_feature 1..18: note = synthetic
  source 1..18: mol_type = other DNA
cagagcattagcagcttt

SEQ ID NO: 92 - protein, 6 aa, synthetic construct
  REGION 1..6: note = synthetic
QSISSF

SEQ ID NO: 93-94 - skipped (2 entries)

SEQ ID NO: 95 - DNA, 24 bp, synthetic construct
  misc_feature 1..24: note = synthetic
  source 1..24: mol_type = other DNA
caacagagttacagttccatcacc

SEQ ID NO: 96 - protein, 8 aa, synthetic construct
  REGION 1..8: note = synthetic
QQSYSSIT

SEQ ID NO: 97 - DNA, 375 bp, synthetic construct
  misc_feature 1..375: note = synthetic
  source 1..375: mol_type = other DNA
caggtgcagctggtggagtctgggggaggcgtggtccagcctgggaggtccctgagactctcctgtgcagcgtctggattcaccttcagtagttatggcatccactgggtccgccaggctccaggcaagtggctggagtgggtggcatttatatggtttgatggaagtaataaatactatgcagactccgtgaagggccgattcaccatctccagagacgattccaagaacacgctgtatctgcaaatgaacagcctgagagccgaggacacggctgtttattactgtgcgagagatggagagatttttggagtgcttatttcctctgatgcttttgatatctggggccaagggacaatggtcaccgtctcttca

SEQ ID NO: 98 - protein, 125 aa, synthetic construct
  REGION 1..125: note = synthetic
QVQLVESGGGVVQPGRSLRLSCAASGFTFSSYGIHWVRQAPGKWLEWVAFIWFDGSNKYYADSVKGRFTISRDDSKNTLYLQMNSLRAEDTAVYYCARDGEIFGVLISSDAFDIWGQGTMVTVSS

SEQ ID NO: 99 - DNA, 24 bp, synthetic construct
  misc_feature 1..24: note = synthetic
  source 1..24: mol_type = other DNA
ggattcaccttcagtagttatggc

SEQ ID NO: 100 - protein, 8 aa, synthetic construct
  REGION 1..8: note = synthetic
GFTFSSYG

SEQ ID NO: 101 - DNA, 24 bp, synthetic construct
  misc_feature 1..24: note = synthetic
  source 1..24: mol_type = other DNA
atatggtttgatggaagtaataaa

SEQ ID NO: 102 - protein, 8 aa, synthetic construct
  REGION 1..8: note = synthetic
IWFDGSNK

SEQ ID NO: 103 - DNA, 54 bp, synthetic construct
  misc_feature 1..54: note = synthetic
  source 1..54: mol_type = other DNA
gcgagagatggagagatttttggagtgcttatttcctctgatgcttttgatatc

SEQ ID NO: 104 - protein, 18 aa, synthetic construct
  REGION 1..18: note = synthetic
ARDGEIFGVLISSDAFDI

SEQ ID NO: 105 - DNA, 321 bp, synthetic construct
  misc_feature 1..321: note = synthetic
  source 1..321: mol_type = other DNA
gacatccagatgacccagtctccatcctccctgtctgcatctgtaggagacagagtcaccatcacttgccgggcaagtcggggcattagaaatgatttaggctggtttcagcagaaaccagggaaagcccctaagcgcctgatctatgttgcatccaatttgcaaagtggggtcccatcaaggttcagcggcagtggatctgggacagaattcactctcacaatcagcagcctgcagcctgaagattttgcaacttattactgtctacagcataatagttacccgatcaccttcggccaagggacacgactggagattaaa

SEQ ID NO: 106 - protein, 107 aa, synthetic construct
  REGION 1..107: note = synthetic
DIQMTQSPSSLSASVGDRVTITCRASRGIRNDLGWFQQKPGKAPKRLIYVASNLQSGVPSRFSGSGSGTEFTLTISSLQPEDFATYYCLQHNSYPITFGQGTRLEIK

SEQ ID NO: 107 - DNA, 18 bp, synthetic construct
  misc_feature 1..18: note = synthetic
  source 1..18: mol_type = other DNA
cggggcattagaaatgat

SEQ ID NO: 108 - protein, 6 aa, synthetic construct
  REGION 1..6: note = synthetic
RGIRND

SEQ ID NO: 109-110 - skipped (2 entries)

SEQ ID NO: 111 - DNA, 27 bp, synthetic construct
  misc_feature 1..27: note = synthetic
  source 1..27: mol_type = other DNA
ctacagcataatagttacccgatcacc

SEQ ID NO: 112 - protein, 9 aa, synthetic construct
  REGION 1..9: note = synthetic
LQHNSYPIT

SEQ ID NO: 113 - DNA, 354 bp, synthetic construct
  misc_feature 1..354: note = synthetic
  source 1..354: mol_type = other DNA
gaggtgcagctggtggagtctgggggaggcttggtacagcctggggggtccctgagactctcctgtgcagcctctggattcaccttcagaagctacgacatgcactgggtccgccaaggttcaggaaaaggtctggagtgggtctcagctattggtactgctggtgacacatactatttaggctccgtgaagggccgattcaccatctccagagaaaatgccaagaactccttgtatcttcaaatgaacagcctgagagccggggacacggctgtgtattactgtgcaagagcgtggttcggggacgtattcctggactactggggccagggaaccctggtcaccgtctcctca

SEQ ID NO: 114 - protein, 118 aa, synthetic construct
  REGION 1..118: note = synthetic
EVQLVESGGGLVQPGGSLRLSCAASGFTFRSYDMHWVRQGSGKGLEWVSAIGTAGDTYYLGSVKGRFTISRENAKNSLYLQMNSLRAGDTAVYYCARAWFGDVFLDYWGQGTLVTVSS

SEQ ID NO: 115 - DNA, 24 bp, synthetic construct
  misc_feature 1..24: note = synthetic
  source 1..24: mol_type = other DNA
ggattcaccttcagaagctacgac

SEQ ID NO: 116 - protein, 8 aa, synthetic construct
  REGION 1..8: note = synthetic
GFTFRSYD

SEQ ID NO: 117 - DNA, 21 bp, synthetic construct
  misc_feature 1..21: note = synthetic
  source 1..21: mol_type = other DNA
attggtactgctggtgacaca

SEQ ID NO: 118 - protein, 7 aa, synthetic construct
  REGION 1..7: note = synthetic
IGTAGDT

SEQ ID NO: 119 - DNA, 36 bp, synthetic construct
  misc_feature 1..36: note = synthetic
  source 1..36: mol_type = other DNA
gcaagagcgtggttcggggacgtattcctggactac

SEQ ID NO: 120 - protein, 12 aa, synthetic construct
  REGION 1..12: note = synthetic
ARAWFGDVFLDY

SEQ ID NO: 121 - DNA, 318 bp, synthetic construct
  misc_feature 1..318: note = synthetic
  source 1..318: mol_type = other DNA
gaaatagtgatgacgcagtctccagccaccctgtctgtgtctccaggggaaagagccaccctctcctgcagggccagtcagagtgttagcagcaacttagcctggtaccagcagaaacctggccaggctcccaggctcctcatatatggtgcatccaccagggccactggtatcccagccaggttcagtggcagtgggtctgggacagagttcactctcaccatcagcagcctgcagtctgaagattttgcaggctattactgtcagcagtataataacaggctgactttcggcggagggaccaaggtggagatcaaa

SEQ ID NO: 122 - protein, 106 aa, synthetic construct
  REGION 1..106: note = synthetic
EIVMTQSPATLSVSPGERATLSCRASQSVSSNLAWYQQKPGQAPRLLIYGASTRATGIPARFSGSGSGTEFTLTISSLQSEDFAGYYCQQYNNRLTFGGGTKVEIK

SEQ ID NO: 123 - DNA, 18 bp, synthetic construct
  misc_feature 1..18: note = synthetic
  source 1..18: mol_type = other DNA
cagagtgttagcagcaac

SEQ ID NO: 124 - protein, 6 aa, synthetic construct
  REGION 1..6: note = synthetic
QSVSSN

SEQ ID NO: 125-126 - skipped (2 entries)

SEQ ID NO: 127 - DNA, 24 bp, synthetic construct
  misc_feature 1..24: note = synthetic
  source 1..24: mol_type = other DNA
cagcagtataataacaggctgact

SEQ ID NO: 128 - protein, 8 aa, synthetic construct
  REGION 1..8: note = synthetic
QQYNNRLT

SEQ ID NO: 129 - DNA, 381 bp, synthetic construct
  misc_feature 1..381: note = synthetic
  source 1..381: mol_type = other DNA
gaggtgcagctggtggagtctgggggaggcttggtccagcctggagggtccctgagactctcctgtgcagcctctggattcaccttcagtgaccactacatggtctgggtccgccaggctccagggaaggggctggagtgggttggccgtactagaaacaaagctaatagttatagcacagaatatgccgcgtctgtgaaaggcagattcaccatctcaagagatgattcaaagaagtcactgtatctgcaaatgaacagcctgaaaaccgaggacacggccgtgtattactgtgctagagggggggaaacactatggttcggggagtccaactacggtatggacgtctggggccaagggaccacggtcaccgtctcctca

SEQ ID NO: 130 - protein, 127 aa, synthetic construct
  REGION 1..127: note = synthetic
EVQLVESGGGLVQPGGSLRLSCAASGFTFSDHYMVWVRQAPGKGLEWVGRTRNKANSYSTEYAASVKGRFTISRDDSKKSLYLQMNSLKTEDTAVYYCARGGETLWFGESNYGMDVWGQGTTVTVSS

SEQ ID NO: 131 - DNA, 24 bp, synthetic construct
  misc_feature 1..24: note = synthetic
  source 1..24: mol_type = other DNA
ggattcaccttcagtgaccactac

SEQ ID NO: 132 - protein, 8 aa, synthetic construct
  REGION 1..8: note = synthetic
GFTFSDHY

SEQ ID NO: 133 - DNA, 30 bp, synthetic construct
  misc_feature 1..30: note = synthetic
  source 1..30: mol_type = other DNA
actagaaacaaagctaatagttatagcaca

SEQ ID NO: 134 - protein, 10 aa, synthetic construct
  REGION 1..10: note = synthetic
TRNKANSYST

SEQ ID NO: 135 - DNA, 54 bp, synthetic construct
  misc_feature 1..54: note = synthetic
  source 1..54: mol_type = other DNA
gctagagggggggaaacactatggttcggggagtccaactacggtatggacgtc

SEQ ID NO: 136 - protein, 18 aa, synthetic construct
  REGION 1..18: note = synthetic
ARGGETLWFGESNYGMDV

SEQ ID NO: 137 - DNA, 324 bp, synthetic construct
  misc_feature 1..324: note = synthetic
  source 1..324: mol_type = other DNA
gaaattgtgttgacgcagtctccagacaccctgtctttgtctccaggggaaagagccaccctctcctgcagggccagtcagagtgttagcagcacctacttagcctggtaccagcagaaacctggccaggctcccagtctcctcatctatggtgcatccagcagggccactggcatcccagacaggttcagtggcagcgggtctgggacagacttcactctcaccatcagcagactggagcctgaagattttgcagtgtattactgtcagcagtatggtaggtcacctctcactttcggcggagggaccaaggtggagatcaaa

SEQ ID NO: 138 - protein, 108 aa, synthetic construct
  REGION 1..108: note = synthetic
EIVLTQSPDTLSLSPGERATLSCRASQSVSSTYLAWYQQKPGQAPSLLIYGASSRATGIPDRFSGSGSGTDFTLTISRLEPEDFAVYYCQQYGRSPLTFGGGTKVEIK

SEQ ID NO: 139 - DNA, 21 bp, synthetic construct
  misc_feature 1..21: note = synthetic
  source 1..21: mol_type = other DNA
cagagtgttagcagcacctac

SEQ ID NO: 140 - protein, 7 aa, synthetic construct
  REGION 1..7: note = synthetic
QSVSSTY

SEQ ID NO: 141-142 - skipped (2 entries)

SEQ ID NO: 143 - DNA, 27 bp, synthetic construct
  misc_feature 1..27: note = synthetic
  source 1..27: mol_type = other DNA
cagcagtatggtaggtcacctctcact

SEQ ID NO: 144 - protein, 9 aa, synthetic construct
  REGION 1..9: note = synthetic
QQYGRSPLT

SEQ ID NO: 145 - DNA, 348 bp, synthetic construct
  misc_feature 1..348: note = synthetic
  source 1..348: mol_type = other DNA
caggtgcagctggtggagtctgggggaggcgtggtccagcctgggaggtccctgagactctcctgtgcagcgtctggcttcaccttcaataactatggcatgcactgggtccgccaggctccaggcatggggctggagtgggtggcagttatatggcacgatggaagtgataaatactatgcagactccgtgaagggccgattcaccatctccagagacaattccaagaacacgctgtatctgcaaatgaacagcctgagagccgaggacacggctgtgtattactgtgcgagaaattggaacctctttgactactggggccagggaaccctggtcactgtctcctca

SEQ ID NO: 146 - protein, 116 aa, synthetic construct
  REGION 1..116: note = synthetic
QVQLVESGGGVVQPGRSLRLSCAASGFTFNNYGMHWVRQAPGMGLEWVAVIWHDGSDKYYADSVKGRFTISRDNSKNTLYLQMNSLRAEDTAVYYCARNWNLFDYWGQGTLVTVSS

SEQ ID NO: 147 - DNA, 24 bp, synthetic construct
  misc_feature 1..24: note = synthetic
  source 1..24: mol_type = other DNA
ggcttcaccttcaataactatggc

SEQ ID NO: 148 - protein, 8 aa, synthetic construct
  REGION 1..8: note = synthetic
GFTFNNYG

SEQ ID NO: 149 - DNA, 24 bp, synthetic construct
  misc_feature 1..24: note = synthetic
  source 1..24: mol_type = other DNA
atatggcacgatggaagtgataaa

SEQ ID NO: 150 - protein, 8 aa, synthetic construct
  REGION 1..8: note = synthetic
IWHDGSDK

SEQ ID NO: 151 - DNA, 27 bp, synthetic construct
  misc_feature 1..27: note = synthetic
  source 1..27: mol_type = other DNA
gcgagaaattggaacctctttgactac

SEQ ID NO: 152 - protein, 9 aa, synthetic construct
  REGION 1..9: note = synthetic
ARNWNLFDY

SEQ ID NO: 153 - DNA, 324 bp, synthetic construct
  misc_feature 1..324: note = synthetic
  source 1..324: mol_type = other DNA
gacatccagatgacccagtctccatcctccctgtctgcatctgtaggagacagaatcaccatcacttgccgggcaagtcagagcatcagcacctatttacattggtatcagcagaaaccagggaaagcccctaagctcctgatctatgctgcatccactttgcagagtggggtcccatcaaggttcagtggcagtggatctgggacagatttcactctcaccatcagcagtctgcaacctgaagattttgcaacttactactgtcaacagagtttcagtacccctccgataaacttcggccaagggaccaagctggagatcaaa

SEQ ID NO: 154 - protein, 108 aa, synthetic construct
  REGION 1..108: note = synthetic
DIQMTQSPSSLSASVGDRITITCRASQSISTYLHWYQQKPGKAPKLLIYAASTLQSGVPSRFSGSGSGTDFTLTISSLQPEDFATYYCQQSFSTPPINFGQGTKLEIK

SEQ ID NO: 155 - DNA, 18 bp, synthetic construct
  misc_feature 1..18: note = synthetic
  source 1..18: mol_type = other DNA
cagagcatcagcacctat

SEQ ID NO: 156 - protein, 6 aa, synthetic construct
  REGION 1..6: note = synthetic
QSISTY

SEQ ID NO: 157-158 - skipped (2 entries)

SEQ ID NO: 159 - DNA, 30 bp, synthetic construct
  misc_feature 1..30: note = synthetic
  source 1..30: mol_type = other DNA
caacagagtttcagtacccctccgataaac

SEQ ID NO: 160 - protein, 10 aa, synthetic construct
  REGION 1..10: note = synthetic
QQSFSTPPIN

SEQ ID NO: 161 - DNA, 384 bp, synthetic construct
  misc_feature 1..384: note = synthetic
  source 1..384: mol_type = other DNA
gaggtgcagctggtggagtctgggggaggcttggtccagcctggggggtccctgagactctcctgtgcagcctctaaattcacctttgacacctttgccatgagctgggtccgccaggctccagggaaggggttggaatgggtctcatttattagtagttctggtggtcgcacagactatgtagactccgtgaagggccggttcaccatctccagagacaattccaagaacaccctgtatctgcaaatgaacagcctgcgagccgaggacacggccgtatattactgtgcgaaagaacggacgatttttggagtgcttattctgggccccgacaactacggtatggacgtctggggccaagggaccacggtcaccgtctcctca

SEQ ID NO: 162 - protein, 128 aa, synthetic construct
  REGION 1..128: note = synthetic
EVQLVESGGGLVQPGGSLRLSCAASKFTFDTFAMSWVRQAPGKGLEWVSFISSSGGRTDYVDSVKGRFTISRDNSKNTLYLQMNSLRAEDTAVYYCAKERTIFGVLILGPDNYGMDVWGQGTTVTVSS

SEQ ID NO: 163 - DNA, 24 bp, synthetic construct
  misc_feature 1..24: note = synthetic
  source 1..24: mol_type = other DNA
aaattcacctttgacacctttgcc

SEQ ID NO: 164 - protein, 8 aa, synthetic construct
  REGION 1..8: note = synthetic
KFTFDTFA

SEQ ID NO: 165 - DNA, 24 bp, synthetic construct
  misc_feature 1..24: note = synthetic
  source 1..24: mol_type = other DNA
attagtagttctggtggtcgcaca

SEQ ID NO: 166 - protein, 8 aa, synthetic construct
  REGION 1..8: note = synthetic
ISSSGGRT

SEQ ID NO: 167 - DNA, 63 bp, synthetic construct
  misc_feature 1..63: note = synthetic
  source 1..63: mol_type = other DNA
gcgaaagaacggacgatttttggagtgcttattctgggccccgacaactacggtatggacgtc

SEQ ID NO: 168 - protein, 21 aa, synthetic construct
  REGION 1..21: note = synthetic
AKERTIFGVLILGPDNYGMDV

SEQ ID NO: 169 - DNA, 324 bp, synthetic construct
  misc_feature 1..324: note = synthetic
  source 1..324: mol_type = other DNA
gacatccagatgacccagtctccatcctccctgtctgcatttgtaggagacagagtcaccatcacttgccgggcaagtcagagcattagcacctatttaaattggtatcagcaaaaaccagggaaagcccctaaactcctgatctatgctgcatccagtttgcaaagtggggtctcatcaaggttcagtggcagtggatctgggacagatttcactctcaccatcagcagtctgcaacctgaagattttgcaacttactactgtcaacagagttacagtgcccctccgatcaccttcggccaagggacacgactggagattaaa

SEQ ID NO: 170 - protein, 108 aa, synthetic construct
  REGION 1..108: note = synthetic
DIQMTQSPSSLSAFVGDRVTITCRASQSISTYLNWYQQKPGKAPKLLIYAASSLQSGVSSRFSGSGSGTDFTLTISSLQPEDFATYYCQQSYSAPPITFGQGTRLEIK

SEQ ID NO: 171 - DNA, 18 bp, synthetic construct
  misc_feature 1..18: note = synthetic
  source 1..18: mol_type = other DNA
cagagcattagcacctat

SEQ ID NO: 172 - protein, 6 aa, synthetic construct
  REGION 1..6: note = synthetic
QSISTY

SEQ ID NO: 173-174 - skipped (2 entries)

SEQ ID NO: 175 - DNA, 30 bp, synthetic construct
  misc_feature 1..30: note = synthetic
  source 1..30: mol_type = other DNA
caacagagttacagtgcccctccgatcacc

SEQ ID NO: 176 - protein, 10 aa, synthetic construct
  REGION 1..10: note = synthetic
QQSYSAPPIT

SEQ ID NO: 177 - DNA, 384 bp, synthetic construct
  misc_feature 1..384: note = synthetic
  source 1..384: mol_type = other DNA
caggtacagctgcagcagtcaggtccaggactggtgaagccctcgcagaccctctcactcacctgtgccatctccggggacagtgtctctagcaacattcctgcttggaactggatcaggcagtccccttcgagaggccttgagtggctgggaaggacatactacaggtccaagtggtataatgattatgcagtatctgtgaaaagtcgaataaccatcaatccagacacatccaagaaccacttctccctgcagctgaactctgtgactcccgaggacacggctgtgtattactgtgcaagaggaagggtctatgacaggtcttctaggtacttctacgctatggacgtctggggccaagggaccacggtcaccgtctcctca

SEQ ID NO: 178 - protein, 128 aa, synthetic construct
  REGION 1..128: note = synthetic
QVQLQQSGPGLVKPSQTLSLTCAISGDSVSSNIPAWNWIRQSPSRGLEWLGRTYYRSKWYNDYAVSVKSRITINPDTSKNHFSLQLNSVTPEDTAVYYCARGRVYDRSSRYFYAMDVWGQGTTVTVSS

SEQ ID NO: 179 - DNA, 30 bp, synthetic construct
  misc_feature 1..30: note = synthetic
  source 1..30: mol_type = other DNA
ggggacagtgtctctagcaacattcctgct

SEQ ID NO: 180 - protein, 10 aa, synthetic construct
  REGION 1..10: note = synthetic
GDSVSSNIPA

SEQ ID NO: 181 - DNA, 27 bp, synthetic construct
  misc_feature 1..27: note = synthetic
  source 1..27: mol_type = other DNA
acatactacaggtccaagtggtataat

SEQ ID NO: 182 - protein, 9 aa, synthetic construct
  REGION 1..9: note = synthetic
TYYRSKWYN

SEQ ID NO: 183 - DNA, 54 bp, synthetic construct
  misc_feature 1..54: note = synthetic
  source 1..54: mol_type = other DNA
gcaagaggaagggtctatgacaggtcttctaggtacttctacgctatggacgtc

SEQ ID NO: 184 - protein, 18 aa, synthetic construct
  REGION 1..18: note = synthetic
ARGRVYDRSSRYFYAMDV

SEQ ID NO: 185 - DNA, 324 bp, synthetic construct
  misc_feature 1..324: note = synthetic
  source 1..324: mol_type = other DNA
gacatccagatgacccagtctccatcctccctgtctgcatctgtaggagacagagtcaccatcacttgccgggcaagtcagagcattagcagctatttaaattggtatcagcagaaaccagggaaagcccctaagctcctgatctatgctgcatccagtttgcaaagtggggtcccatcaaggttcagtggcagtggatctgggacagatttcactctcaccatcagcagtctgcaacctgaagattttgcaacttactactgtcaacagagttacagtaattatccgatcaccttcggccaagggacacgactggagattaaa

SEQ ID NO: 186 - protein, 108 aa, synthetic construct
  REGION 1..108: note = synthetic
DIQMTQSPSSLSASVGDRVTITCRASQSISSYLNWYQQKPGKAPKLLIYAASSLQSGVPSRFSGSGSGTDFTLTISSLQPEDFATYYCQQSYSNYPITFGQGTRLEIK

SEQ ID NO: 187 - DNA, 18 bp, synthetic construct
  misc_feature 1..18: note = synthetic
  source 1..18: mol_type = other DNA
cagagcattagcagctat

SEQ ID NO: 188 - protein, 6 aa, synthetic construct
  REGION 1..6: note = synthetic
QSISSY

SEQ ID NO: 189-190 - skipped (2 entries)

SEQ ID NO: 191 - DNA, 30 bp, synthetic construct
  misc_feature 1..30: note = synthetic
  source 1..30: mol_type = other DNA
caacagagttacagtaattatccgatcacc

SEQ ID NO: 192 - protein, 10 aa, synthetic construct
  REGION 1..10: note = synthetic
QQSYSNYPIT

SEQ ID NO: 193 - DNA, 357 bp, synthetic construct
  misc_feature 1..357: note = synthetic
  source 1..357: mol_type = other DNA
gaggtgcagctggtggagtctgggggaggcttggttcagccgggggggtccctgagactctcctgtgcagcctctggattcaccttcagaacctacgacatgcactgggtccgccaagctacaggaaaaggtctggagtgggtctcagctattggtactgctggtgacacatactatccaggctccgtgaagggccgattcaccatctccagagaaaatgccaagaactccttgtatcttcaaatgaacagcctgagagccggtgacacggctgtgtattactgtgcacgaacgatttttggagtggttcttacctttgactactggggccagggaaccctggtcaccgtctcctca

SEQ ID NO: 194 - protein, 119 aa, synthetic construct
  REGION 1..119: note = synthetic
EVQLVESGGGLVQPGGSLRLSCAASGFTFRTYDMHWVRQATGKGLEWVSAIGTAGDTYYPGSVKGRFTISRENAKNSLYLQMNSLRAGDTAVYYCARTIFGVVLTFDYWGQGTLVTVSS

SEQ ID NO: 195 - DNA, 24 bp, synthetic construct
  misc_feature 1..24: note = synthetic
  source 1..24: mol_type = other DNA
ggattcaccttcagaacctacgac

SEQ ID NO: 196 - protein, 8 aa, synthetic construct
  REGION 1..8: note = synthetic
GFTFRTYD

SEQ ID NO: 197 - DNA, 21 bp, synthetic construct
  misc_feature 1..21: note = synthetic
  source 1..21: mol_type = other DNA
attggtactgctggtgacaca

SEQ ID NO: 198 - protein, 7 aa, synthetic construct
  REGION 1..7: note = synthetic
IGTAGDT

SEQ ID NO: 199 - DNA, 39 bp, synthetic construct
  misc_feature 1..39: note = synthetic
  source 1..39: mol_type = other DNA
gcacgaacgatttttggagtggttcttacctttgactac

SEQ ID NO: 200 - protein, 13 aa, synthetic construct
  REGION 1..13: note = synthetic
ARTIFGVVLTFDY

SEQ ID NO: 201 - DNA, 324 bp, synthetic construct
  misc_feature 1..324: note = synthetic
  source 1..324: mol_type = other DNA
gacatccagatgacccagtctccatcctccctgtctgcatctgtaggagacagagtcaccatcacttgccgggcaagtcagagcattagcagctctttaaattggtatcagcagaaaccagggaaagcccctaagctcctgatctatgctgcatccagtttgcacagtggggtcccatcaaggttcagtggcagtggatctgggacagatttcactctcaccatcagcagtctgcaacctgaagattttgcaacttactactgtcaacagacttacagtatccctccgaccaccttcggccaagggaccaaggtggaaatcaaa

SEQ ID NO: 202 - protein, 108 aa, synthetic construct
  REGION 1..108: note = synthetic
DIQMTQSPSSLSASVGDRVTITCRASQSISSSLNWYQQKPGKAPKLLIYAASSLHSGVPSRFSGSGSGTDFTLTISSLQPEDFATYYCQQTYSIPPTTFGQGTKVEIK

SEQ ID NO: 203 - DNA, 18 bp, synthetic construct
  misc_feature 1..18: note = synthetic
  source 1..18: mol_type = other DNA
cagagcattagcagctct

SEQ ID NO: 204 - protein, 6 aa, synthetic construct
  REGION 1..6: note = synthetic
QSISSS

SEQ ID NO: 205-206 - skipped (2 entries)

SEQ ID NO: 207 - DNA, 30 bp, synthetic construct
  misc_feature 1..30: note = synthetic
  source 1..30: mol_type = other DNA
caacagacttacagtatccctccgaccacc

SEQ ID NO: 208 - protein, 10 aa, synthetic construct
  REGION 1..10: note = synthetic
QQTYSIPPTT

SEQ ID NO: 209 - DNA, 384 bp, synthetic construct
  misc_feature 1..384: note = synthetic
  source 1..384: mol_type = other DNA
gaggtgcagctggtggagtctgggggaggcttggtacagcctggggggtccctgagactctcctgtgcagcctctggattcacctttagcaactatgccatgatctgggtccgccaggctccagggaaggggctggagtgggtctcaggtattagtggtagtggtggcagtatatactacgcagactccgtgaagggccggttcaccatctccagagacaattccaagaacacgctgtatctgcaaatgaacagcctgagagccgaggacacggccgtatattactgtgcgaaagaaggaattattagtatggttcggggacttatcaactactaccacggtatggacgtctggggccaagggaccacggtcaccgtctcctca

SEQ ID NO: 210 - protein, 128 aa, synthetic construct
  REGION 1..128: note = synthetic
EVQLVESGGGLVQPGGSLRLSCAASGFTFSNYAMIWVRQAPGKGLEWVSGISGSGGSIYYADSVKGRFTISRDNSKNTLYLQMNSLRAEDTAVYYCAKEGIISMVRGLINYYHGMDVWGQGTTVTVSS

SEQ ID NO: 211 - DNA, 24 bp, synthetic construct
  misc_feature 1..24: note = synthetic
  source 1..24: mol_type = other DNA
ggattcacctttagcaactatgcc

SEQ ID NO: 212 - protein, 8 aa, synthetic construct
  REGION 1..8: note = synthetic
GFTFSNYA

SEQ ID NO: 213 - DNA, 24 bp, synthetic construct
  misc_feature 1..24: note = synthetic
  source 1..24: mol_type = other DNA
attagtggtagtggtggcagtata

SEQ ID NO: 214 - protein, 8 aa, synthetic construct
  REGION 1..8: note = synthetic
ISGSGGSI

SEQ ID NO: 215 - DNA, 63 bp, synthetic construct
  misc_feature 1..63: note = synthetic
  source 1..63: mol_type = other DNA
gcgaaagaaggaattattagtatggttcggggacttatcaactactaccacggtatggacgtc

SEQ ID NO: 216 - protein, 21 aa, synthetic construct
  REGION 1..21: note = synthetic
AKEGIISMVRGLINYYHGMDV

SEQ ID NO: 217 - DNA, 324 bp, synthetic construct
  misc_feature 1..324: note = synthetic
  source 1..324: mol_type = other DNA
gaaattgtgttgacgcagtctccaggcaccctgtctttgtctccaggggaaagagccaccctctcctgcagggccagtcagagtgttagcagcagctacttagcctggtaccagcagaaacctggccaggctcccaggctcctcatctatggtgcatccagcagggccactggcatcccagacaggttcagtggcagtgggtctgggacagacttcactctcaccatcagcagactggagcctgaagattttgcagtgtattactgtcagcagtatggtagctcaccttggacgttcggccaagggaccaaggtggaaatcaaa

SEQ ID NO: 218 - protein, 108 aa, synthetic construct
  REGION 1..108: note = synthetic
EIVLTQSPGTLSLSPGERATLSCRASQSVSSSYLAWYQQKPGQAPRLLIYGASSRATGIPDRFSGSGSGTDFTLTISRLEPEDFAVYYCQQYGSSPWTFGQGTKVEIK

SEQ ID NO: 219 - DNA, 21 bp, synthetic construct
  misc_feature 1..21: note = synthetic
  source 1..21: mol_type = other DNA
cagagtgttagcagcagctac

SEQ ID NO: 220 - protein, 7 aa, synthetic construct
  REGION 1..7: note = synthetic
QSVSSSY

SEQ ID NO: 221-222 - skipped (2 entries)

SEQ ID NO: 223 - DNA, 27 bp, synthetic construct
  misc_feature 1..27: note = synthetic
  source 1..27: mol_type = other DNA
cagcagtatggtagctcaccttggacg

SEQ ID NO: 224 - protein, 9 aa, synthetic construct
  REGION 1..9: note = synthetic
QQYGSSPWT

SEQ ID NO: 225 - DNA, 360 bp, synthetic construct
  misc_feature 1..360: note = synthetic
  source 1..360: mol_type = other DNA
caggtgcagctggtgcagtctggggctgaggtgaagaagcctggggcctcagtgaaggtttcctgcaaggcatctggatacaccttcaccagctactatatgcactgggtgcgacaggcccctggacaagggcttgagtggttgggaataatcaaccctagtggtggtagcacaagctacgcacagaagttccagggcagagtcaccatgaccagggacacgtccacgagcacagtctacatggagctgagcagcctgagatctgaggacacggccgtgtattactgtgcgagagagacaggagaagctggtgaggtttttaactactggggccagggaacccaggtcaccgtctcctca

SEQ ID NO: 226 - protein, 120 aa, synthetic construct
  REGION 1..120: note = synthetic
QVQLVQSGAEVKKPGASVKVSCKASGYTFTSYYMHWVRQAPGQGLEWLGIINPSGGSTSYAQKFQGRVTMTRDTSTSTVYMELSSLRSEDTAVYYCARETGEAGEVFNYWGQGTQVTVSS

SEQ ID NO: 227 - DNA, 24 bp, synthetic construct
  misc_feature 1..24: note = synthetic
  source 1..24: mol_type = other DNA
ggatacaccttcaccagctactat

SEQ ID NO: 228 - protein, 8 aa, synthetic construct
  REGION 1..8: note = synthetic
GYTFTSYY

SEQ ID NO: 229 - DNA, 24 bp, synthetic construct
  misc_feature 1..24: note = synthetic
  source 1..24: mol_type = other DNA
atcaaccctagtggtggtagcaca

SEQ ID NO: 230 - protein, 8 aa, synthetic construct
  REGION 1..8: note = synthetic
INPSGGST

SEQ ID NO: 231 - DNA, 39 bp, synthetic construct
  misc_feature 1..39: note = synthetic
  source 1..39: mol_type = other DNA
gcgagagagacaggagaagctggtgaggtttttaactac

SEQ ID NO: 232 - protein, 13 aa, synthetic construct
  REGION 1..13: note = synthetic
ARETGEAGEVFNY

SEQ ID NO: 233 - DNA, 324 bp, synthetic construct
  misc_feature 1..324: note = synthetic
  source 1..324: mol_type = other DNA
gacatccagatgacccagtctccatcctccctgtctgcatctgtaggagacagagtcaccatcacttgccgggcaagtcagatcattagcaggtatttaaattggtatcagcataaaccagggaaagcccctaaggtcctgatctatgctgcctccactttgcaaagtggggtcccatcaaggttcagtggcagtggatctgggacagatttcactctcaccatcagcagtctgcaacctgaagattttgcaacttactactgtcaacagagttacagtacccctccgatcaccttcggccaagggacacgactggagattaaa

SEQ ID NO: 234 - protein, 108 aa, synthetic construct
  REGION 1..108: note = synthetic
DIQMTQSPSSLSASVGDRVTITCRASQIISRYLNWYQHKPGKAPKVLIYAASTLQSGVPSRFSGSGSGTDFTLTISSLQPEDFATYYCQQSYSTPPITFGQGTRLEIK

SEQ ID NO: 235 - DNA, 18 bp, synthetic construct
  misc_feature 1..18: note = synthetic
  source 1..18: mol_type = other DNA
cagatcattagcaggtat

SEQ ID NO: 236 - protein, 6 aa, synthetic construct
  REGION 1..6: note = synthetic
QIISRY

SEQ ID NO: 237-238 - skipped (2 entries)

SEQ ID NO: 239 - DNA, 30 bp, synthetic construct
  misc_feature 1..30: note = synthetic
  source 1..30: mol_type = other DNA
caacagagttacagtacccctccgatcacc

SEQ ID NO: 240 - protein, 10 aa, synthetic construct
  REGION 1..10: note = synthetic
QQSYSTPPIT

SEQ ID NO: 241 - DNA, 381 bp, synthetic construct
  misc_feature 1..381: note = synthetic
  source 1..381: mol_type = other DNA
gaggtgcagctggtggagtctgggggaggcttggtacagcctggagggtccctgagactctcctgtgcagcctctggattcaccttcagtagttatgaaatgaactgggtccgccaggctccagggaaggggctggagtgggtttcatacattggtagtagtggtcgtgccacatactacgcagactctgtgaagggccgattcaccatctccagagacaacgccaaaaactcactgtatctgcaaatgaacagcctgagagccgaggacacggctgtttattactgtgcgagaccttcgagcatagcagctctgttacggaaccagtaccacttcggtatggacgtctggggccaagggaccacggtcaccgtctcctca

SEQ ID NO: 242 - protein, 127 aa, synthetic construct
  REGION 1..127: note = synthetic
EVQLVESGGGLVQPGGSLRLSCAASGFTFSSYEMNWVRQAPGKGLEWVSYIGSSGRATYYADSVKGRFTISRDNAKNSLYLQMNSLRAEDTAVYYCARPSSIAALLRNQYHFGMDVWGQGTTVTVSS

SEQ ID NO: 243 - DNA, 24 bp, synthetic construct
  misc_feature 1..24: note = synthetic
  source 1..24: mol_type = other DNA
ggattcaccttcagtagttatgaa

SEQ ID NO: 244 - protein, 8 aa, synthetic construct
  REGION 1..8: note = synthetic
GFTFSSYE

SEQ ID NO: 245 - DNA, 24 bp, synthetic construct
  misc_feature 1..24: note = synthetic
  source 1..24: mol_type = other DNA
attggtagtagtggtcgtgccaca

SEQ ID NO: 246 - protein, 8 aa, synthetic construct
  REGION 1..8: note = synthetic
IGSSGRAT

SEQ ID NO: 247 - DNA, 60 bp, synthetic construct
  misc_feature 1..60: note = synthetic
  source 1..60: mol_type = other DNA
gcgagaccttcgagcatagcagctctgttacggaaccagtaccacttcggtatggacgtc

SEQ ID NO: 248 - protein, 20 aa, synthetic construct
  REGION 1..20: note = synthetic
ARPSSIAALLRNQYHFGMDV

SEQ ID NO: 249 - DNA, 324 bp, synthetic construct
  misc_feature 1..324: note = synthetic
  source 1..324: mol_type = other DNA
gacatccagatgacccagtctccatcctccctgtctgcatctgtaggagacagagtcaccatcacttgccgggcaagtcagagcattaccagctatttaaattggtatcagcagaaaccagggaaagcccctaagctcctgatctatgctgcatccagtttgcaaggtggggtcccatcaaggttcagtggcagtggatctgggacagatttcactctcaccatcagcagtctgcaacctgaagattttgcaacttactactgtcaacagagttacagtacccctccgatcaccttcggccaagggacacgactggagattaaa

SEQ ID NO: 250 - protein, 108 aa, synthetic construct
  REGION 1..108: note = synthetic
DIQMTQSPSSLSASVGDRVTITCRASQSITSYLNWYQQKPGKAPKLLIYAASSLQGGVPSRFSGSGSGTDFTLTISSLQPEDFATYYCQQSYSTPPITFGQGTRLEIK

SEQ ID NO: 251 - DNA, 18 bp, synthetic construct
  misc_feature 1..18: note = synthetic
  source 1..18: mol_type = other DNA
cagagcattaccagctat

SEQ ID NO: 252 - protein, 6 aa, synthetic construct
  REGION 1..6: note = synthetic
QSITSY

SEQ ID NO: 253-254 - skipped (2 entries)

SEQ ID NO: 255 - DNA, 30 bp, synthetic construct; identical to SEQ ID NO: 239
  misc_feature 1..30: note = synthetic
  source 1..30: mol_type = other DNA

SEQ ID NO: 256 - protein, 10 aa, synthetic construct
  REGION 1..10: note = synthetic
QQSYSTPPIT

SEQ ID NO: 257 - DNA, 360 bp, synthetic construct
  misc_feature 1..360: note = synthetic
  source 1..360: mol_type = other DNA
caggtgcagctggtgcagtctggggctgaggtgaagaagcctggggcctcagtgaaggtttcctgcaaggcatctggatacaccttcaccagctactatatgcactgggtgcgacaggcccctggacaagggcttgagtggatgggaataatcaaccctagtggtggtagcacaagctacgcacagaagttccagggcagagtcaccatgaccagggacacgtccacgagcacagtctacatggagctgagcagcctgagatctgaggacacggccgtgtattactgtgcgagagagataggagaagctggtgaagtttttaactactggggccagggaaccctggtcaccgtctcctca

SEQ ID NO: 258 - protein, 120 aa, synthetic construct
  REGION 1..120: note = synthetic
QVQLVQSGAEVKKPGASVKVSCKASGYTFTSYYMHWVRQAPGQGLEWMGIINPSGGSTSYAQKFQGRVTMTRDTSTSTVYMELSSLRSEDTAVYYCAREIGEAGEVFNYWGQGTLVTVSS

SEQ ID NO: 259 - DNA, 24 bp, synthetic construct
  misc_feature 1..24: note = synthetic
  source 1..24: mol_type = other DNA
ggatacaccttcaccagctactat

SEQ ID NO: 260 - protein, 8 aa, synthetic construct
  REGION 1..8: note = synthetic
GYTFTSYY

SEQ ID NO: 261 - DNA, 24 bp, synthetic construct
  misc_feature 1..24: note = synthetic
  source 1..24: mol_type = other DNA
atcaaccctagtggtggtagcaca

SEQ ID NO: 262 - protein, 8 aa, synthetic construct
  REGION 1..8: note = synthetic
INPSGGST

SEQ ID NO: 263 - DNA, 39 bp, synthetic construct
  misc_feature 1..39: note = synthetic
  source 1..39: mol_type = other DNA
gcgagagagataggagaagctggtgaagtttttaactac

SEQ ID NO: 264 - protein, 13 aa, synthetic construct
  REGION 1..13: note = synthetic
AREIGEAGEVFNY

SEQ ID NO: 265 - DNA, 324 bp, synthetic construct
  misc_feature 1..324: note = synthetic
  source 1..324: mol_type = other DNA
gacatccagatgacccagtctccatcctccctgtctgcatctgtaggagacagagtcaccatcacttgccgggcaagtcagagcattagcaggtatttaaattggtatcagcataaaccagggaaagcccctaaggtcctgatctatgctgcatccattttgcaaagtggggtcccatcaaggttcagtggcagtggatctgggacagatttcactctcaccatcagcagtctgcaacctgaagattttgcaacttactactgtcaacagagttacagtacccctccgatcaccttcggccaagggacacgactggagattaaa

SEQ ID NO: 266 - protein, 108 aa, synthetic construct
  REGION 1..108: note = synthetic
DIQMTQSPSSLSASVGDRVTITCRASQSISRYLNWYQHKPGKAPKVLIYAASILQSGVPSRFSGSGSGTDFTLTISSLQPEDFATYYCQQSYSTPPITFGQGTRLEIK

SEQ ID NO: 267 - DNA, 18 bp, synthetic construct
  misc_feature 1..18: note = synthetic
  source 1..18: mol_type = other DNA
cagagcattagcaggtat

SEQ ID NO: 268 - protein, 6 aa, synthetic construct
  REGION 1..6: note = synthetic
QSISRY

SEQ ID NO: 269-270 - skipped (2 entries)

SEQ ID NO: 271 - DNA, 30 bp, synthetic construct; identical to SEQ ID NO: 239
  misc_feature 1..30: note = synthetic
  source 1..30: mol_type = other DNA

SEQ ID NO: 272 - protein, 10 aa, synthetic construct
  REGION 1..10: note = synthetic
QQSYSTPPIT

SEQ ID NO: 273 - DNA, 381 bp, synthetic construct
  misc_feature 1..381: note = synthetic
  source 1..381: mol_type = other DNA
gaggtgcagctggtggagtctgggggaggcttggtacagcctggagggtccctgagactctcctgtgcagcctctggattcaccttcagtacttatgaaatgaactgggtccgccaggctccagggaaggggctggagtgggtttcatatagtagtagtagtggtagaaccatatactacgcagactctgtgaagggccgattcaccatctccagagacaacgccaagaactcactgtttctgcaaatgaacagcctgagagccgaggacacggctgtttattactgtgcgagaccttcgagtatagagactctgttacggaatcagtaccactacggtgtggacgtctggggccaagggaccacggtcaccgtctcctca

SEQ ID NO: 274 - protein, 127 aa, synthetic construct
  REGION 1..127: note = synthetic
EVQLVESGGGLVQPGGSLRLSCAASGFTFSTYEMNWVRQAPGKGLEWVSYSSSSGRTIYYADSVKGRFTISRDNAKNSLFLQMNSLRAEDTAVYYCARPSSIETLLRNQYHYGVDVWGQGTTVTVSS

SEQ ID NO: 275 - DNA, 24 bp, synthetic construct
  misc_feature 1..24: note = synthetic
  source 1..24: mol_type = other DNA
ggattcaccttcagtacttatgaa

SEQ ID NO: 276 - protein, 8 aa, synthetic construct
  REGION 1..8: note = synthetic
GFTFSTYE

SEQ ID NO: 277 - DNA, 24 bp, synthetic construct
  misc_feature 1..24: note = synthetic
  source 1..24: mol_type = other DNA
agtagtagtagtggtagaaccata

SEQ ID NO: 278 - protein, 8 aa, synthetic construct
  REGION 1..8: note = synthetic
SSSSGRTI

SEQ ID NO: 279 - DNA, 60 bp, synthetic construct
  misc_feature 1..60: note = synthetic
  source 1..60: mol_type = other DNA
gcgagaccttcgagtatagagactctgttacggaatcagtaccactacggtgtggacgtc

SEQ ID NO: 280 - protein, 20 aa, synthetic construct
  REGION 1..20: note = synthetic
ARPSSIETLLRNQYHYGVDV

SEQ ID NO: 281 - DNA, 324 bp, synthetic construct
  misc_feature 1..324: note = synthetic
  source 1..324: mol_type = other DNA
gacatccagatgacccagtctccatcctccctgtctgcatctgtaggagacagagtcaccatcacttgccgggcaagtcagagcattagcagctatttaaattggtatcagcagaaaccagggaaagcccctaagctcctgatctatgctgcatccagtttgcaaagtggggtcccgtcaaggttcagtggcagtggatctgggacagatttcactctcaccatcagcagtctgcaacctgaagattttgcaacttactactgtcaacagagttacagtacccctccgatcaccttcggccaagggacacgactggagattaaa

SEQ ID NO: 282 - protein, 108 aa, synthetic construct
  REGION 1..108: note = synthetic
DIQMTQSPSSLSASVGDRVTITCRASQSISSYLNWYQQKPGKAPKLLIYAASSLQSGVPSRFSGSGSGTDFTLTISSLQPEDFATYYCQQSYSTPPITFGQGTRLEIK

SEQ ID NO: 283 - DNA, 18 bp, synthetic construct
  misc_feature 1..18: note = synthetic
  source 1..18: mol_type = other DNA
cagagcattagcagctat

SEQ ID NO: 284 - protein, 6 aa, synthetic construct
  REGION 1..6: note = synthetic
QSISSY

SEQ ID NO: 285-286 - skipped (2 entries)

SEQ ID NO: 287 - DNA, 30 bp, synthetic construct; identical to SEQ ID NO: 239
  misc_feature 1..30: note = synthetic
  source 1..30: mol_type = other DNA

SEQ ID NO: 288 - protein, 10 aa, synthetic construct
  REGION 1..10: note = synthetic
QQSYSTPPIT

SEQ ID NO: 289 - DNA, 384 bp, synthetic construct
  misc_feature 1..384: note = synthetic
  source 1..384: mol_type = other DNA
gaggtgcagctggtggagtctgggggaggcttggcacagcctggagggtccctgagactctcctgtgcagcctctggattcaccttcagtagtcatgaaatgaactgggtccgccaggctccagggaaggggctggagtgggtttcatacattagtcgtagtggtagaatcataaactacgcagactctgtgaagggccgattcaccatctccagagacaacgccaagaactcactgtatctgcaaatgaacagcctgagagccgaggacacggctgtttattactgtgcgagagagagaggctcgtattacgatattttgactggttcccaggactacggtatggacgtctggggccaagggaccacggtcaccgtctcctca

SEQ ID NO: 290 - protein, 128 aa, synthetic construct
  REGION 1..128: note = synthetic
EVQLVESGGGLAQPGGSLRLSCAASGFTFSSHEMNWVRQAPGKGLEWVSYISRSGRIINYADSVKGRFTISRDNAKNSLYLQMNSLRAEDTAVYYCARERGSYYDILTGSQDYGMDVWGQGTTVTVSS

SEQ ID NO: 291 - DNA, 24 bp, synthetic construct
  misc_feature 1..24: note = synthetic
  source 1..24: mol_type = other DNA
ggattcaccttcagtagtcatgaa

SEQ ID NO: 292 - protein, 8 aa, synthetic construct
  REGION 1..8: note = synthetic
GFTFSSHE

SEQ ID NO: 293 - DNA, 24 bp, synthetic construct
  misc_feature 1..24: note = synthetic
  source 1..24: mol_type = other DNA
attagtcgtagtggtagaatcata

SEQ ID NO: 294 - protein, 8 aa, synthetic construct
  REGION 1..8: note = synthetic
ISRSGRII

SEQ ID NO: 295 - DNA, 63 bp, synthetic construct
  misc_feature 1..63: note = synthetic
  source 1..63: mol_type = other DNA
gcgagagagagaggctcgtattacgatattttgactggttcccaggactacggtatggacgtc

SEQ ID NO: 296 - protein, 21 aa, synthetic construct
  REGION 1..21: note = synthetic
ARERGSYYDILTGSQDYGMDV

SEQ ID NO: 297 - DNA, 324 bp, synthetic construct
  misc_feature 1..324: note = synthetic
  source 1..324: mol_type = other DNA
gacatccagatgacccagtctccatcctccctgtctgcatctgtaggagacagagtcaccatcacttgccgggcaagtcagaccattagcacctatttaaattggtatcagcagaaaccagggaaagcccctaagctcctgatctatgctgcatccagtttgcaaagtggggtcccatcaaggttcagtggcagtggatctgggacagatttcactctcaccatcagcagtctgcaacctgaagattttgcaacttactactgtcaacagagttacagtacccctccgatcaccttcggccaagggacacgactggagattaaa

SEQ ID NO: 298 - protein, 108 aa, synthetic construct
  REGION 1..108: note = synthetic
DIQMTQSPSSLSASVGDRVTITCRASQTISTYLNWYQQKPGKAPKLLIYAASSLQSGVPSRFSGSGSGTDFTLTISSLQPEDFATYYCQQSYSTPPITFGQGTRLEIK

SEQ ID NO: 299 - DNA, 18 bp, synthetic construct
  misc_feature 1..18: note = synthetic
  source 1..18: mol_type = other DNA
cagaccattagcacctat

SEQ ID NO: 300 - protein, 6 aa, synthetic construct
  REGION 1..6: note = synthetic
QTISTY

SEQ ID NO: 301-302 - skipped (2 entries)

SEQ ID NO: 303 - DNA, 30 bp, synthetic construct; identical to SEQ ID NO: 239
  misc_feature 1..30: note = synthetic
  source 1..30: mol_type = other DNA

SEQ ID NO: 304 - protein, 10 aa, synthetic construct
  REGION 1..10: note = synthetic
QQSYSTPPIT

SEQ ID NO: 305 - DNA, 381 bp, synthetic construct
  misc_feature 1..381: note = synthetic
  source 1..381: mol_type = other DNA
gaggtgcagctggtggagtctgggggaggcttggtacagcctggagggtccctgagactctcctgtgcagcctctggattcaccttcagtagttatgaaatgaactgggtccgccaggctccagggaaggggctggagtgggtttcatacattagtagtagtggtagtaccaaatactacgcagactctgtgaagggccgattcaccatctccagagacaacgccaagaactcactgtatctgcaaatgaacagcctgagagccgaggacacggctgtttattactgtgcgagaccttcgagtataccagctctgttacggaaccagtaccactacggtatggacgtctggggccaagggaccacggtcaccgtctcctca

SEQ ID NO: 306 - protein, 127 aa, synthetic construct
  REGION 1..127: note = synthetic
EVQLVESGGGLVQPGGSLRLSCAASGFTFSSYEMNWVRQAPGKGLEWVSYISSSGSTKYYADSVKGRFTISRDNAKNSLYLQMNSLRAEDTAVYYCARPSSIPALLRNQYHYGMDVWGQGTTVTVSS

SEQ ID NO: 307 - DNA, 24 bp, synthetic construct
  misc_feature 1..24: note = synthetic
  source 1..24: mol_type = other DNA
ggattcaccttcagtagttatgaa

SEQ ID NO: 308 - protein, 8 aa, synthetic construct
  REGION 1..8: note = synthetic
GFTFSSYE

SEQ ID NO: 309 - DNA, 24 bp, synthetic construct
  misc_feature 1..24: note = synthetic
  source 1..24: mol_type = other DNA
attagtagtagtggtagtaccaaa

SEQ ID NO: 310 - protein, 8 aa, synthetic construct
  REGION 1..8: note = synthetic
ISSSGSTK

SEQ ID NO: 311 - DNA, 60 bp, synthetic construct
  misc_feature 1..60: note = synthetic
  source 1..60: mol_type = other DNA
gcgagaccttcgagtataccagctctgttacggaaccagtaccactacggtatggacgtc

SEQ ID NO: 312 - protein, 20 aa, synthetic construct
  REGION 1..20: note = synthetic
ARPSSIPALLRNQYHYGMDV

SEQ ID NO: 313 - DNA, 2051 bp, Zaire ebolavirus
  source 1..2051: mol_type = genomic DNA
gaattcgccaccatgggcgtgaccggcatcctgcagctgccccgggacagattcaagcggaccagcttcttcctgtgggtcatcatcctgttccagcggaccttcagcatccccctgggcgtgatccacaacagcaccctgcaggtgtccgacgtggacaagctcgtgtgccgggacaagctgagcagcaccaaccagctgagaagcgtgggcctgaacctggaaggcaatggcgtggccaccgatgtgcctagcgccaccaagagatggggcttcagatccggcgtgccccccaaggtcgtgaattatgaggccggcgagtgggccgagaactgctacaacctggaaatcaagaagcccgacggcagcgagtgcctgcctgctgcccctgatggcatcagaggcttcccccggtgcagatacgtgcacaaggtgtccggcacaggcccctgcgctggcgatttcgcctttcacaaagagggcgcctttttcctgtacgaccggctggcctccaccgtgatctacagaggcaccacctttgccgagggcgtggtggcctttctgatcctgcctcaggccaagaaggacttcttcagcagccaccccctgcgcgagcctgtgaatgccacagaggatcccagcagcggctactacagcaccaccatcagataccaggccaccggcttcggcaccaacgagacagagtacctgttcgaggtggacaacctgacctacgtgcagctggaaagccggttcaccccccagtttctgctgcagctgaacgagacaatctacgccagcggcaagcggagcaacaccaccggcaagctgatctggaaagtgaaccccgagatcgataccacaatcggagagtgggccttctgggagacaaagaagaacctgacccggaagatcagaagcgaggaactgagcttcaccgccgtgtccaacggccccaagaacatcagcggacagagccccgccagaaccagcagcgaccccgagacaaacaccaccaatgaggaccacaagatcatggccagcgagaacagcagcgccatggtgcaggtgcacagccagggaagaaaggccgctgtgtcccacctgaccaccctggccacaatctccaccagccctcagagcctgaccacaaagcctggccccgacaactccacccacaacacccccgtgtacaagctggacatcagcgaggccacacaagtgggccagcaccacagaagggccgacaacgatagcaccgccagcgatacccctccagccacaactgctgccggacctctgaaggccgagaataccaacaccagcaagagcgccgacagcctggatctggccaccaccacaagcccccagaactactctgagacagccggcaacaacaacacccaccaccaggataccggcgaggaaagcgccagctctggcaagctgggactgatcaccaacacaatcgccggcgtggccggcctgattaccggggggagaagaaccagacgggaagtgatcgtgaacgcccagcccaagtgcaaccccaacctgcactactggaccacccaggatgagggcgctgctatcggactggcctggatcccttactttggccctgccgccgagggcatctacaccgagggactgatgcacaaccaggacggcctgatctgcggactgaggcagctggccaacgaaaccacacaggctctgcagctgttcctgagagccaccaccgagctgaggaccttctccatcctgaacagaaaggctatcgacttcctgctgcagcgctggggcggcacctgtcacattctgggccctgactgctgcatcgagccccacgactggaccaagaatatcaccgacaagatcgaccagatcatccacgactttgtggacaagaccctgcccgaccagggcgacaatgacaactggtggacaggctggcggcagtggattcctgccggcattggagtgaccggcgtgatcattgccgtgatcgccctgttctgcatctgcaagttcgtgttctgagcggccgc

SEQ ID NO: 314 - protein, 676 aa, Zaire ebolavirus
MGVTGILQLPRDRFKRTSFFLWVIILFQRTFSIPLGVIHNSTLQVSDVDKLVCRDKLSSTNQLRSVGLNLEGNGVATDVPSATKRWGFRSGVPPKVVNYEAGEWAENCYNLEIKKPDGSECLPAAPDGIRGFPRCRYVHKVSGTGPCAGDFAFHKEGAFFLYDRLASTVIYRGTTFAEGVVAFLILPQAKKDFFSSHPLREPVNATEDPSSGYYSTTIRYQATGFGTNETEYLFEVDNLTYVQLESRFTPQFLLQLNETIYASGKRSNTTGKLIWKVNPEIDTTIGEWAFWETKKNLTRKIRSEELSFTAVSNGPKNISGQSPARTSSDPETNTTNEDHKIMASENSSAMVQVHSQGRKAAVSHLTTLATISTSPQPPTTKTGPDNSTHNTPVYKLDISEATQVGQHHRRADNDSTASDTPPATTAAGPLKAENTNTSKSADSLDLATTTSPQNYSETAGNNNTHHQDTGEESASSGKLGLITNTIAGVAGLITGGRRTRREVIVNAQPKCNPNLHYWTTQDEGAAIGLAWIPYFGPAAEGIYTEGLMHNQDGLICGLRQLANETTQALQLFLRATTELRTFSILNRKAIDFLLQRWGGTCHILGPDCCIEPHDWTKNITDKIDQIIHDFVDKTLPDQGDNDNWWTGWRQWIPAGIGVTGVIIAVIALFCICKFVF

SEQ ID NO: 315 - protein, 676 aa, Zaire ebolavirus; identical to SEQ ID NO: 314

SEQ ID NO: 316 - protein, 364 aa, Zaire ebolavirus
MGVTGILQLPRDRFKRTSFFLWVIILFQRTFSIPLGVIHNSTLQVSDVDKLVCRDKLSSTNQLRSVGLNLEGNGVATDVPSATKRWGFRSGVPPKVVNYEAGEWAENCYNLEIKKPDGSECLPAAPDGIRGFPRCRYVHKVSGTGPCAGDFAFHKEGAFFLYDRLASTVIYRGTTFAEGVVAFLILPQAKKDFFSSHPLREPVNATEDPSSGYYSTTIRYQATGFGTNETEYLFEVDNLTYVQLESRFTPQFLLQLNETIYASGKRSNTTGKLIWKVNPEIDTTIGEWAFWETKKTSLEKFAVKSCLSQLYQTDPKTSVVRVRRELLPTQRPTQQMKTTKSWLQKIPLQWFKCTVKEGKLQCRI

SEQ ID NO: 317 - protein, 360 aa, synthetic construct
  REGION 1..360: note = aa 1-332: Zaire_Ebola_GP aa 33 through 364 of AHX24650 aa 333-360: myc-myc-hexahistidine tag
IPLGVIHNSTLQVSDVDKLVCRDKLSSTNQLRSVGLNLEGNGVATDVPSATKRWGFRSGVPPKVVNYEAGEWAENCYNLEIKKPDGSECLPAAPDGIRGFPRCRYVHKVSGTGPCAGDFAFHKEGAFFLYDRLASTVIYRGTTFAEGVVAFLILPQAKKDFFSSHPLREPVNATEDPSSGYYSTTIRYQATGFGTNETEYLFEVDNLTYVQLESRFTPQFLLQLNETIYASGKRSNTTGKLIWKVNPEIDTTIGEWAFWETKKTSLEKFAVKSCLSQLYQTDPKTSVVRVRRELLPTQRPTQQMKTTKSWLQKIPLQWFKCTVKEGKLQCRIEQKLISEEDLGGEQKLISEEDLHHHHHH

SEQ ID NO: 318 - protein, 628 aa, synthetic construct
  REGION 1..628: note = aa 1-618: Zaire ebolavirus (strain H.sapiens-wt/GIN/2014/Kissidougou-C15) GP (aa 33 through 650 (AHX24649.1)) aa 619-628: decahistidine tag
IPLGVIHNSTLQVSDVDKLVCRDKLSSTNQLRSVGLNLEGNGVATDVPSATKRWGFRSGVPPKVVNYEAGEWAENCYNLEIKKPDGSECLPAAPDGIRGFPRCRYVHKVSGTGPCAGDFAFHKEGAFFLYDRLASTVIYRGTTFAEGVVAFLILPQAKKDFFSSHPLREPVNATEDPSSGYYSTTIRYQATGFGTNETEYLFEVDNLTYVQLESRFTPQFLLQLNETIYTSGKRSNTTGKLIWKVNPEIDTTIGEWAFWETKKNLTRKIRSEELSFTVVSNGAKNISGQSPARTSSDPGTNTTTEDHKIMASENSSAMVQVHSQGREAAVSHLTTLATISTSPQSLTTKPGPDNSTHNTPVYKLDISEATQVEQHHRRTDNDSTASDTPSATTAAGPPKAENTNTSKSTDFLDPATTTSPQNHSETAGNNNTHHQDTGEESASSGKLGLITNTIAGVAGLITGGRRTRREAIVNAQPKCNPNLHYWTTQDEGAAIGLAWIPYFGPAAEGIYIEGLMHNQDGLICGLRQLANETTQALQLFLRATTELRTFSILNRKAIDFLLQRWGGTCHILGPDCCIEPHDWTKNITDKIDQIIHDFVDKTLPDQGDNDNWWTGWRQHHHHHHHHHH